European Patent Specification EP 3 914 704 B9, published October 4, 2023. Title: A METHOD FOR SCREENING OF AN IN VITRO DISPLAY LIBRARY WITHIN A CELL. Applicant: Vipergen ApS. The sequence listing filed with the application follows.

SEQUENCE LISTING (4 sequences)

SEQ ID NO: 1 - DNA, 20 bp, Artificial Sequence
  Primer
aaagctgggagacaccaatg

SEQ ID NO: 2 - DNA, 20 bp, Artificial Sequence
  Primer
ttggtgtctcccagctttga

SEQ ID NO: 3 - DNA, 58 bp, Artificial Sequence
  Primer
agcactaagccttgatggccacattcctacttctccctaaggtgcagttttgccaagg

SEQ ID NO: 4 - DNA, 60 bp, Artificial Sequence
  Primer
ccttggcaaaactgcaccttagggagaagtaggaatgtggccatcaaggcttagtgctca